European Patent Application EP 4 455 299 A1, published October 30, 2024. Title: METHOD FOR GENERATING LABELED NUCLEIC ACID MOLECULAR POPULATION AND KIT THEREOF. Applicant: BGI SHENZHEN. The sequence listing filed with the application follows.

SEQUENCE LISTING (14 sequences)

SEQ ID NO: 1 - DNA, 171 bp, Artificial Sequence
  Nucleotide sequence of DNA library molecule
  misc_feature (26)..(42): n=a, t, c or g
  misc_feature (75)..(99): n=a, t, c or g
  misc_feature (138)..(154): n=a, t, c or g
gaacgacatggctacgatccgacttnnnnnnnnnnnnnnnnnaagtcggaggccaagcggtcttaggaagacaannnnnnnnnnnnnnnnnnnnnnnnnctgataaggtcgccatgcctctcagtacgtcagcagttnnnnnnnnnnnnnnnnncaactccttggctcaca

SEQ ID NO: 2 - DNA, 24 bp, Artificial Sequence
  Nucleotide sequence of DNB primer
gccatgtcgttcggaaccgagtgt

SEQ ID NO: 3 - DNA, 36 bp, Artificial Sequence
  Nucleotide sequence of chip sequence synthesis primer
ctgctgacgtactgagaggcatggcgaccttatcag

SEQ ID NO: 4 - DNA, 36 bp, Artificial Sequence; identical to SEQ ID NO: 3
  Consensus sequence X1

SEQ ID NO: 5 - DNA, 13 bp, Artificial Sequence
  Consensus sequence X2
ttgtcttcctaag

SEQ ID NO: 6 - DNA, 54 bp, Artificial Sequence
  Nucleotide sequence of polyT primer
  misc_feature (16)..(25): n=a, t, c or g
  misc_feature (54)..(54): v=a, g or c
accgcttggcctccgnnnnnnnnnnttttttttttttttttttttttttttttv

SEQ ID NO: 7 - DNA, 30 bp, Artificial Sequence
  TSO sequence
  misc_feature (28)..(29): ribonucleotide
aagcagtggtatcaacgcagagtacatggg

SEQ ID NO: 8 - DNA, 74 bp, Artificial Sequence
  Chip sequence
  misc_feature (37)..(61): n=a, t, c or g
ctgctgacgtactgagaggcatggcgaccttatcagnnnnnnnnnnnnnnnnnnnnnnnnnttgtcttcctaag

SEQ ID NO: 9 - DNA, 24 bp, Artificial Sequence
  Bridging oligonucleotide sequence
aggccaagcggtcttaggaagaca

SEQ ID NO: 10 - DNA, 23 bp, Artificial Sequence
  Sequence of cDNA amplification primer 1
ctgctgacgtactgagaggcatg

SEQ ID NO: 11 - DNA, 25 bp, Artificial Sequence
  Sequence of cDNA amplification primer 2
aagcagtggtatcaacgcagagtac

SEQ ID NO: 12 - DNA, 22 bp, Artificial Sequence
  Library construction primer 1
ctgctgacgtactgagaggcat

SEQ ID NO: 13 - DNA, 24 bp, Artificial Sequence
  Library construction primer 2
gagacgttctcgactcagaagatg

SEQ ID NO: 14 - DNA, 24 bp, Artificial Sequence
  Primer sequence to prepare DNB for sequencing
ggcctccgacttgagacgttctcg